European Patent Application EP 4 763 861 A1, published June 24, 2026. Title: An engineered cell comprising an anti-CD19 and anti-CD20 chimeric antigen receptor, a nucleic acid or vector, a kit and their use. Applicant: AvenCell Therapeutics Inc. Application EP. The sequence listing filed with the application follows.

SEQUENCE LISTING (70 sequences)

SEQ ID NO: 1 - protein, 8 aa, Mus musculus
GVSLPDYG

SEQ ID NO: 2 - protein, 7 aa, Mus musculus
IWGSETT

SEQ ID NO: 3 - protein, 14 aa, Mus musculus
AKHYYYGGSYAMDY

SEQ ID NO: 4 - protein, 6 aa, Mus musculus
QDISKY

SEQ ID NO: 5 - protein, 9 aa, Mus musculus
QQGNTLPYT

SEQ ID NO: 6 - protein, 245 aa, Mus musculus
DIQMTQTTSSLSASLGDRVTISCRASQDISKYLNWYQQKPDGTVKLLIYHTSRLHSGVPSRFSGSGSGTDYSLTISNLEQEDIATYFCQQGNTLPYTFGGGTKLEITGSTSGSGKPGSGEGSTKGEVKLQESGPGLVAPSQSLSVTCTVSGVSLPDYGVSWIRQPPRKGLEWLGVIWGSETTYYNSALKSRLTIIKDNSKSQVFLKMNSLQTDDTAIYYCAKHYYYGGSYAMDYWGQGTSVTVSS

SEQ ID NO: 7 - protein, 10 aa, Lama glama
GRTFSNYNMG

SEQ ID NO: 8 - protein, 18 aa, Lama glama
AIDWSGGSPYYAASVRGR

SEQ ID NO: 9 - protein, 12 aa, Lama glama
PLSYGSTWLADY

SEQ ID NO: 10 - protein, 121 aa, Lama glama
QVQLVESGGGLVQPGGSLRLSCAASGRTFSNYNMGWFRQAPGQGLEFVAAIDWSGGSPYYAASVRGRFTISRDNSKNTLYLQMNSLRAEDTAVYYCAAPLSYGSTWLADYWGQGTLVTVSS

SEQ ID NO: 11 - protein, 5 aa, synthetic construct
  source 1..5: note = linker sequence
GGGGS

SEQ ID NO: 12 - protein, 25 aa, synthetic construct
  source 1..25: note = linker sequence
GGGGSGGGGSGASAAGGGGSGGGGS

SEQ ID NO: 13 - protein, 25 aa, synthetic construct
  source 1..25: note = linker sequence
GGGGSGGGGSGGGGSGGGGSGGGGS

SEQ ID NO: 14 - protein, 18 aa, synthetic construct
  source 1..18: note = linker sequence
GSTSGSGKPGSGEGSTKG

SEQ ID NO: 15 - protein, 44 aa, Homo sapiens
TTTPAPRPPTPAPTIASQPLSLRPEACRPAAGGAVHTRGLDFAC

SEQ ID NO: 16 - protein, 54 aa, Homo sapiens
FVPVFLPAKPTTTPAPRPPTPAPTIASQPLSLRPEACRPAAGGAVHTRGLDFAC

SEQ ID NO: 17 - protein, 39 aa, Homo sapiens
IEVMYPPPYLDNEKSNGTIIHVKGKHLCPSPLFPGPSKP

SEQ ID NO: 18 - protein, 133 aa, synthetic construct
  source 1..133: note = CD28 extracellular hinge domain
KILVKQSPMLVAYDNAVNLSCKYSYNLFSREFRASLHKGLDSAVEVCVVYGNYSQQLQVYSKTGFNCDGKLGNESVTFYLQNLYVNQTDIYFCKIEVMAPPPALDNEKSNGTIIHVKGKHLCPSPLFPGPSKP

SEQ ID NO: 19 - protein, 12 aa, synthetic construct
  source 1..12: note = IgG4 extracellular hinge domain
ESKYGPPCPPCP

SEQ ID NO: 20 - protein, 15 aa, Homo sapiens
EPKSCDKTHTCPPCP

SEQ ID NO: 21 - protein, 12 aa, Homo sapiens
ERKCCVECPPCP

SEQ ID NO: 22 - protein, 25 aa, Homo sapiens
DIYIWAPLAGTCGVLLLSLVITLYC

SEQ ID NO: 23 - protein, 21 aa, Homo sapiens
IYIWAPLAGTCGVLLLSLVIT

SEQ ID NO: 24 - protein, 28 aa, Homo sapiens
MFWVLVVVGGVLACYSLLVTVAFIIFWV

SEQ ID NO: 25 - protein, 27 aa, Homo sapiens
FWVLVVVGGVLACYSLLVTVAFIIFWV

SEQ ID NO: 26 - protein, 21 aa, Homo sapiens
FWLPIGCAAFVVVCILGCILI

SEQ ID NO: 27 - protein, 22 aa, Homo sapiens
MALIVLGGVAGLLLFIGLGIFF

SEQ ID NO: 28 - protein, 112 aa, Homo sapiens
RVKFSRSADAPAYQQGQNQLYNELNLGRREEYDVLDKRRGRDPEMGGKPRRKNPQEGLYNELQKDKMAEAYSEIGMKGERRRGKGHDGLYQGLSTATKDTYDALHMQALPPR

SEQ ID NO: 29 - protein, 48 aa, Homo sapiens
QRRKYRSNKGESPVEPAEPCHYSCPREEEGSTIPIQEDYRKPEPACSP

SEQ ID NO: 30 - protein, 41 aa, Homo sapiens
RSKRSRLLHSDYMNMTPRRPGPTRKHYQPYAPPRDFAAYRS

SEQ ID NO: 31 - protein, 41 aa, synthetic construct
  source 1..41: note = CD28 intracellular signaling domain
RSKRSRGGHSDYMNMTPRRPGPTRKHYQPYAPPRDFAAYRS

SEQ ID NO: 32 - protein, 42 aa, Homo sapiens
ALYLLRRDQRLPPDAHKPPGGGSFRTPIQEEQADAHSTLAKI

SEQ ID NO: 33 - protein, 42 aa, Homo sapiens
KRGRKKLLYIFKQPFMRPVQTTQEEDGCSCRFPEEEEGGCEL

SEQ ID NO: 34 - protein, 42 aa, synthetic construct
  source 1..42: note = 4-1BB intracellular signaling domain
KRGRKKGGYIFKQPFMRPVQTTQEEDGCSCRFPEEEEGGCEL

SEQ ID NO: 35 - protein, 38 aa, Homo sapiens
CWLTKKKYSSSVHDPNGEYMFMRAVNTAKKSRLTDVTL

SEQ ID NO: 36 - protein, 24 aa, Homo sapiens
LCARPRRSPAQEDGKVYINMPGRG

SEQ ID NO: 37 - protein, 52 aa, Homo sapiens
YFLGRLVPRGRGAAEAATRKQRITETESPYQELQGQRSDVYSDLNTQRPYYK

SEQ ID NO: 38 - protein, 97 aa, Homo sapiens
CSRAARGTIGARRTGQPLKEDPSAVPVFSVDYGELDFQWREKTPEPPVPCVPEQTEYATIVFPSGMGTSSPARRGSADGPRSAQPLRPEDGHCSWPL

SEQ ID NO: 39 - protein, 41 aa, Homo sapiens
AVSLSKMLKKRSPLTTGVYVKMPPTEPECEKQFQPYFIPIN

SEQ ID NO: 40 - protein, 20 aa, Homo sapiens
  VARIANT 16: note = Xaa can be alanine or serine
LEKEALKKIIEDQQEXLNKW

SEQ ID NO: 41 - protein, 20 aa, Homo sapiens
LEKEALKKIIEDQQEALNKW

SEQ ID NO: 42 - protein, 22 aa, Homo sapiens
MDMRVPAQLLGLLLLWLRGARC

SEQ ID NO: 43 - protein, 20 aa, synthetic construct
  source 1..20: note = signal peptide
MRRMQLLLLIALSLALVTNS

SEQ ID NO: 44 - protein, 21 aa, Homo sapiens
MKWKALFTAAILQAQLPITEA

SEQ ID NO: 45 - protein, 22 aa, Homo sapiens
MLLLVTSLLLCELPHPAFLLIP

SEQ ID NO: 46 - protein, 21 aa, Homo sapiens
MALPVTALLLPLALLLHAARP

SEQ ID NO: 47 - DNA, 241 bp, synthetic construct
  source 1..241: mol_type = other DNA; note = promoter
gggcagagcgcacatcgcccacagtccccgagaagttggggggaggggtcggcaattgaaccggtgcctagagaaggtggcgcggggtaaactgggaaagtgatgtcgtgtactggctccgcctttttcccgagggtgggggagaaccgtatataagtgcagtagtcgccgtgaacgttctttttcgcaacgggtttgccgccagaacacagctgaagctcgggatccaccggtcgccacc

SEQ ID NO: 48 - protein, 632 aa, synthetic construct
  source 1..632: note = chimeric antigen receptor
MALPVTALLLPLALLLHAARPQVQLVESGGGLVQPGGSLRLSCAASGRTFSNYNMGWFRQAPGQGLEFVAAIDWSGGSPYYAASVRGRFTISRDNSKNTLYLQMNSLRAEDTAVYYCAAPLSYGSTWLADYWGQGTLVTVSSGGGGSGGGGSGGGGSGGGGSGGGGSDIQMTQTTSSLSASLGDRVTISCRASQDISKYLNWYQQKPDGTVKLLIYHTSRLHSGVPSRFSGSGSGTDYSLTISNLEQEDIATYFCQQGNTLPYTFGGGTKLEITGSTSGSGKPGSGEGSTKGEVKLQESGPGLVAPSQSLSVTCTVSGVSLPDYGVSWIRQPPRKGLEWLGVIWGSETTYYNSALKSRLTIIKDNSKSQVFLKMNSLQTDDTAIYYCAKHYYYGGSYAMDYWGQGTSVTVSSIEVMYPPPYLDNEKSNGTIIHVKGKHLCPSPLFPGPSKPFWVLVVVGGVLACYSLLVTVAFIIFWVKRGRKKLLYIFKQPFMRPVQTTQEEDGCSCRFPEEEEGGCELRVKFSRSADAPAYQQGQNQLYNELNLGRREEYDVLDKRRGRDPEMGGKPRRKNPQEGLYNELQKDKMAEAYSEIGMKGERRRGKGHDGLYQGLSTATKDTYDALHMQALPPR

SEQ ID NO: 49 - protein, 631 aa, synthetic construct
  source 1..631: note = chimeric antigen receptor
MALPVTALLLPLALLLHAARPQVQLVESGGGLVQPGGSLRLSCAASGRTFSNYNMGWFRQAPGQGLEFVAAIDWSGGSPYYAASVRGRFTISRDNSKNTLYLQMNSLRAEDTAVYYCAAPLSYGSTWLADYWGQGTLVTVSSGGGGSGGGGSGGGGSGGGGSGGGGSDIQMTQTTSSLSASLGDRVTISCRASQDISKYLNWYQQKPDGTVKLLIYHTSRLHSGVPSRFSGSGSGTDYSLTISNLEQEDIATYFCQQGNTLPYTFGGGTKLEITGSTSGSGKPGSGEGSTKGEVKLQESGPGLVAPSQSLSVTCTVSGVSLPDYGVSWIRQPPRKGLEWLGVIWGSETTYYNSALKSRLTIIKDNSKSQVFLKMNSLQTDDTAIYYCAKHYYYGGSYAMDYWGQGTSVTVSSIEVMYPPPYLDNEKSNGTIIHVKGKHLCPSPLFPGPSKPFWVLVVVGGVLACYSLLVTVAFIIFWVRSKRSRLLHSDYMNMTPRRPGPTRKHYQPYAPPRDFAAYRSRVKFSRSADAPAYQQGQNQLYNELNLGRREEYDVLDKRRGRDPEMGGKPRRKNPQEGLYNELQKDKMAEAYSEIGMKGERRRGKGHDGLYQGLSTATKDTYDALHMQALPPR

SEQ ID NO: 50 - protein, 634 aa, synthetic construct
  source 1..634: note = chimeric antigen receptor
MALPVTALLLPLALLLHAARPQVQLVESGGGLVQPGGSLRLSCAASGRTFSNYNMGWFRQAPGQGLEFVAAIDWSGGSPYYAASVRGRFTISRDNSKNTLYLQMNSLRAEDTAVYYCAAPLSYGSTWLADYWGQGTLVTVSSGGGGSGGGGSGGGGSGGGGSGGGGSDIQMTQTTSSLSASLGDRVTISCRASQDISKYLNWYQQKPDGTVKLLIYHTSRLHSGVPSRFSGSGSGTDYSLTISNLEQEDIATYFCQQGNTLPYTFGGGTKLEITGSTSGSGKPGSGEGSTKGEVKLQESGPGLVAPSQSLSVTCTVSGVSLPDYGVSWIRQPPRKGLEWLGVIWGSETTYYNSALKSRLTIIKDNSKSQVFLKMNSLQTDDTAIYYCAKHYYYGGSYAMDYWGQGTSVTVSSAAAIEVMYPPPYLDNEKSNGTIIHVKGKHLCPSPLFPGPSKPFWVLVVVGGVLACYSLLVTVAFIIFWVRSKRSRLLHSDYMNMTPRRPGPTRKHYQPYAPPRDFAAYRSRVKFSRSADAPAYQQGQNQLYNELNLGRREEYDVLDKRRGRDPEMGGKPRRKNPQEGLYNELQKDKMAEAYSEIGMKGERRRGKGHDGLYQGLSTATKDTYDALHMQALPPR

SEQ ID NO: 51 - DNA, 1896 bp, synthetic construct
  source 1..1896: mol_type = other DNA; note = chimeric antigen receptor
atggcccttccagtgaccgccctgctgctgccactggctctgctgctgcacgccgctagacctcaggtgcagctggtggaaagcggcgggggcctggtgcagcctggcggcagcctgagactgtcttgcgccgctagcggaagaacttttagcaactacaacatgggctggtttagacaggcccccggccagggcctggagttcgtggctgccatcgactggagcggcggaagcccctattacgccgcctccgtgcggggcagattcaccatcagccgggacaattctaagaataccctgtatctgcaaatgaacagcctgagagccgaagatacagccgtgtactactgcgccgcccctctgagctacggaagcacatggctggccgactactggggacaaggaaccctggtaaccgtctcaagcggcggtggaggatcaggaggtggtggttcaggaggtggaggttctgggggaggcggatctgggggaggaggcagcgacatccagatgacacagacaacctccagcctgagcgccagcctgggcgacagagtgaccatcagctgtagagcctctcaggacatcagcaagtacctgaactggtatcagcagaaacctgatggcaccgtgaagctgctgatctaccacacatctaggctgcactctggagtccccagccggtttagcggaagcgggtcaggcacagactatagcctgaccatctccaatctggaacaggaggacatcgccacctacttctgccagcagggcaacaccctgccttatacattcggtggcggcaccaagctggaaatcaccggcagcacctctggctctggcaagcccggaagcggcgagggctccaccaagggagaggtgaagctgcaggagtccggacctgggctggtggctccaagccagagcctgagcgtgacctgcaccgtgtccggagtgagcctgcctgattacggcgtgtcttggatcagacagcctcctagaaagggactggaatggctgggcgtgatctggggtagcgagacaacatactacaacagcgccctgaagagcagactgacaatcatcaaggacaacagcaaaagccaggtgttcctaaaaatgaactccctgcagaccgacgacaccgccatctactactgtgcgaaacactactactacggcggctcctacgccatggactattggggccagggcaccagcgtgacagtgagcagcatcgaggtgatgtacccccctccttacctggacaacgagaagtccaacggcaccattatccacgtgaaaggcaagcacctgtgccccagccctctgttccccggcccttctaaaccgttctgggttctggtggtcgtgggcggcgtactggcttgctactctctgctggtcacagtggctttcatcatcttctgggtgaaaagaggcagaaagaaactgctgtacatctttaagcagccattcatgcggccagtgcagaccacccaggaggaggacggctgctcttgtcgctttcccgaggaggaggagggcggatgtgagctgagggtgaagtttagcagatccgctgatgcccctgcctatcagcagggacagaaccagctgtacaacgagctgaacctggggagaagagaagagtacgatgtgctggacaagcggagaggcagagatcctgagatgggcggcaagcccagacggaagaatcctcaagagggcctgtacaatgaactgcagaaagacaagatggccgaggcctacagcgagatcggaatgaagggcgagcgcagaagaggcaagggacacgatggactgtaccagggcctgagcaccgccaccaaggatacctatgatgccctgcacatgcaggccctgcctccaaga

SEQ ID NO: 52 - DNA, 1899 bp, synthetic construct
  source 1..1899: mol_type = other DNA; note = chimeric antigen receptor
atggccctgccagtgaccgccctgctgctgcccctggcactgctgctgcacgcagccagaccccaagtgcagctggtggagtcaggcggcgggctagtgcagccaggaggctccctgagactgtcttgcgctgcaagcggcagaaccttctcaaactacaatatggggtggttcaggcaggcccccgggcagggcctggagttcgtggccgctatcgactggagtgggggctccccctactatgcagctagcgtgagaggcagatttaccatctccagagacaactccaagaacactctgtacctccagatgaatagtctgagagccgaagatacagccgtgtactactgtgccgcccccctgagctacggcagcacctggctggctgattactggggtcagggaacactggttacagtgtcatccggaggaggtggtagtggaggcggaggcagtggtggaggcggtagcgggggaggcggatctgggggaggaggcagcgacatccagatgacccagaccacctcctctctgagcgcttcactcggagaccgggtgacaatcagctgtagagcctcccaggatatctctaagtatctgaactggtaccagcagaagccagatggcacagtgaagctgctgatctatcataccagcaggctgcactccggagtgccttccaggttttccggcagcggatccggcaccgattatagcctgaccatctccaatctggagcaggaggacatagcaacctacttttgccagcagggcaataccctgccctacacctttgggggaggaaccaaactcgaaatcaccggctctacttctggaagcggcaagcccggatcaggcgaaggctcaaccaagggcgaggtgaaactgcaggagagcggcccaggactggtcgccccatcacagtccctgtcagtgacctgcaccgttagcggggtgtccctgcctgactacggggtgagctggatcaggcagcctcctcggaagggcctggagtggctgggggtgatctggggctccgagaccacctattataactccgccctgaagtcccggctgaccatcattaaagataacagcaagagccaggtgttcctgaagatgaactcactgcagacagacgacaccgctatctattattgcgccaagcattactactacggcggatcatacgccatggactattggggccagggcacttctgtgaccgtgtcttctatcgaggtgatgtaccccccaccatatctggataacgagaaatccaatggcaccatcattcacgtgaagggcaagcacctgtgtccatctcctctgttccctggcccaagcaagcccttctgggtgctggtggtcgtggggggcgtgctggcctgctactctctgctggtgactgtggcattcatcatcttctgggtgaagcggggcaggaagaaactgctgtacatcttcaagcagccattcatgcggcccgtgcagaccacccaggaagaggatgggtgctcatgccggttccctgaggaggaggagggggggtgcgagctgagggtcaagttttccagaagcgctgacgctcccgcttaccagcagggccaaaatcagctctataacgaactgaatctcggcaggcgcgaggaatatgacgtgctggataagaggcggggacgcgaccctgaaatgggaggaaagcctcggcggaaaaacccacaagaaggactttacaacgaactccaaaaggataagatggctgaagcctactctgagattggcatgaaaggagaacgtcggagaggaaaaggccacgacggactctatcagggactgtctacagccacaaaagacacatacgacgcactccatatgcaggctctcccacctagataa

SEQ ID NO: 53 - DNA, 1893 bp, synthetic construct
  source 1..1893: mol_type = other DNA; note = chimeric antigen receptor
atggccctgccagtgaccgccctgctgctgcccctggcactgctgctgcacgcagccagaccccaagtgcagctggtggagtcaggcggcgggctagtgcagccaggaggctccctgagactgtcttgcgctgcaagcggcagaaccttctcaaactacaatatggggtggttcaggcaggcccccgggcagggcctggagttcgtggccgctatcgactggagtgggggctccccctactatgcagctagcgtgagaggcagatttaccatctccagagacaactccaagaacactctgtacctccagatgaatagtctgagagccgaagatacagccgtgtactactgtgccgcccccctgagctacggcagcacctggctggctgattactggggacagggtacactggttacagtatcatctggcggtggaggatcaggaggtggtggttcaggaggtggaggttctgggggaggcggatctgggggaggaggcagcgacatccagatgacccagaccacctcctctctgagcgcttcactcggagaccgggtgacaatcagctgtagagcctcccaggatatctctaagtatctgaactggtaccagcagaagccagatggcacagtgaagctgctgatctatcataccagcaggctgcactccggagtgccttccaggttttccggcagcggatccggcaccgattatagcctgaccatctccaatctggagcaggaggacatagcaacctacttttgccagcagggcaataccctgccctacacctttgggggaggaaccaaactcgaaatcaccggctctacttctggaagcggcaagcccggatcaggcgaaggctcaaccaagggcgaggtgaaactgcaggagagcggcccaggactggtcgccccatcacagtccctgtcagtgacctgcaccgttagcggggtgtccctgcctgactacggggtgagctggatcaggcagcctcctcggaagggcctggagtggctgggggtgatctggggctccgagaccacctattataactccgccctgaagtcccggctgaccatcattaaagataacagcaagagccaggtgttcctgaagatgaactcactgcagacagacgacaccgctatctattattgcgccaagcattactactacggcggatcatacgccatggactattggggccagggcacttctgtgaccgtgtcttctatcgaggtgatgtaccccccaccatatctggataacgagaaatccaatggcaccatcattcacgtgaagggcaagcacctgtgtccatctcctctgttccctggcccaagcaagcccttctgggtgctggtggtcgtggggggcgtgctggcctgctactctctgctggtgactgtggcattcatcatcttctgggtgagatccaaaaggtctcgcctgctgcacagcgactatatgaatatgacccctcgcaggcctggccctacacgcaagcactatcagccttacgccccccctcgggactttgctgcgtatcggagtagggtgaagtttagcagatccgctgatgcccctgcctatcagcagggacagaaccagctgtacaacgagctgaacctggggagaagagaagagtacgatgtgctggacaagcggagaggcagagatcctgagatgggcggcaagcccagacggaagaatcctcaagagggcctgtacaatgaactgcagaaagacaagatggccgaggcctacagcgagatcggaatgaagggcgagcgcagaagaggcaagggacacgatggactgtaccagggcctgagcaccgccaccaaggatacctatgatgccctgcacatgcaggccctgcctccaaga

SEQ ID NO: 54 - DNA, 1896 bp, synthetic construct
  source 1..1896: mol_type = other DNA; note = chimeric antigen receptor
atggccctgccagtgaccgccctgctgctgcccctggcactgctgctgcacgcagccagaccccaagtgcagctggtggagtcaggcggcgggctagtgcagccaggaggctccctgagactgtcttgcgctgcaagcggcagaaccttctcaaactacaatatggggtggttcaggcaggcccccgggcagggcctggagttcgtggccgctatcgactggagtgggggctccccctactatgcagctagcgtgagaggcagatttaccatctccagagacaactccaagaacactctgtacctccagatgaatagtctgagagccgaagatacagccgtgtactactgtgccgcccccctgagctacggcagcacctggctggctgattactggggacagggtacactggttacagtatcatctggcggtggaggatcaggaggtggtggttcaggaggtggaggttctgggggaggcggatctgggggaggaggcagcgacatccagatgacccagaccacctcctctctgagcgcttcactcggagaccgggtgacaatcagctgtagagcctcccaggatatctctaagtatctgaactggtaccagcagaagccagatggcacagtgaagctgctgatctatcataccagcaggctgcactccggagtgccttccaggttttccggcagcggatccggcaccgattatagcctgaccatctccaatctggagcaggaggacatagcaacctacttttgccagcagggcaataccctgccctacacctttgggggaggaaccaaactcgaaatcaccggctctacttctggaagcggcaagcccggatcaggcgaaggctcaaccaagggcgaggtgaaactgcaggagagcggcccaggactggtcgccccatcacagtccctgtcagtgacctgcaccgttagcggggtgtccctgcctgactacggggtgagctggatcaggcagcctcctcggaagggcctggagtggctgggggtgatctggggctccgagaccacctattataactccgccctgaagtcccggctgaccatcattaaagataacagcaagagccaggtgttcctgaagatgaactcactgcagacagacgacaccgctatctattattgcgccaagcattactactacggcggatcatacgccatggactattggggccagggcacttctgtgaccgtgtcttctatcgaggtgatgtaccccccaccatatctggataacgagaaatccaatggcaccatcattcacgtgaagggcaagcacctgtgtccatctcctctgttccctggcccaagcaagcccttctgggtgctggtggtcgtggggggcgtgctggcctgctactctctgctggtgactgtggcattcatcatcttctgggtgagatccaaaaggtctcgcctgctgcacagcgactatatgaatatgacccctcgcaggcctggccctacacgcaagcactatcagccttacgccccccctcgggactttgctgcgtatcggagtagggtcaagttttccagaagcgctgacgctcccgcttaccagcagggccaaaatcagctctataacgaactgaatctcggcaggcgcgaggaatatgacgtgctggataagaggcggggacgcgaccctgaaatgggaggaaagcctcggcggaaaaacccacaagaaggactttacaacgaactccaaaaggataagatggctgaagcctactctgagattggcatgaaaggagaacgtcggagaggaaaaggccacgacggactctatcagggactgtctacagccacaaaagacacatacgacgcactccatatgcaggctctcccacctagataa

SEQ ID NO: 55 - DNA, 1902 bp, synthetic construct
  source 1..1902: mol_type = other DNA; note = chimeric antigen receptor
atggcccttccagtgaccgccctgctgctgccactggctctgctgctgcacgccgctagacctcaggtgcagctggtggaaagcgggggaggcctggttcagcccggcggcagcctgagactgagctgcgccgctagcggcagaacattcagcaactacaacatgggctggttcagacaagcccctggccagggcctggaattcgtggccgctatcgactggtccggcggcagcccttactacgccgcctccgtgcggggcagattcaccatctctcgggataatagcaagaacaccctctacctgcagatgaatagcctgagagccgaggataccgccgtgtactactgtgccgctcctctgtcttacggcagcacctggctggcagattactggggccagggcaccctggtgacagtgtccagcggcggaggaggcagcggcggaggcggaagcggcggtggtggctctggaggcggcggctccggcggtggcggcagtgatatccagatgacccagaccacttccagcctgtctgcctccctgggcgacagggtgactatcagctgccgcgccagccaggatatttcaaaatacctgaattggtaccagcagaagcccgacggcacagtgaagctgctgatctaccacaccagtcgcctgcacagcggcgtgcccagcaggttcagcggcagcggatccggcacagactacagcctgaccatcagcaacctggagcaggaggatatcgcaacttatttttgccagcagggcaatacactgccttacaccttcggcggcggcaccaagctggaaatcaccggcagcacaagtggctccggcaaaccaggcagcggagagggcagcacaaagggcgaggtgaaactgcaggagagcggccccggcctggtggcccccagccagtctctgagcgtgacctgcaccgtgtccggcgtgtccctgcctgactacggggtgagctggatcaggcagccccccaggaaaggcttggaatggctgggcgtgatctggggcagcgagacaacctattataactctgccctgaagagcagactgaccatcatcaaagacaatagcaaaagccaggtgttcctgaagatgaattcactgcagactgacgatactgccatctattattgtgccaaacactactactatggcggatcctatgccatggattactggggccagggcacctcagtgaccgtgtcctcggccgctgctattgaagtgatgtatccacccccttacctggacaacgagaaatcaaacggcactattatccacgtgaagggaaagcacctgtgcccctcccctctgtttcccggcccaagtaagcccttttgggtgctggtggtggtcgggggcgtgctggcctgttattccctgctggtcacagtggctttcatcatcttctgggtgcgcagcaagaggtccagactgctgcactctgactacatgaacatgactcccaggaggccaggccctactagaaaacactaccagccctacgctcctcctagagacttcgccgcctacaggtccagggtcaagttttccagaagcgctgacgctcccgcttaccagcagggccaaaatcagctctataacgaactgaatctcggcaggcgcgaggaatatgacgtgctggataagaggcggggacgcgaccctgaaatgggaggaaagcctcggcggaaaaacccacaagaaggactttacaacgaactccaaaaggataagatggctgaagcctactctgagattggcatgaaaggagaacgtcggagaggaaaaggccacgacggactctatcagggactgtctacagccacaaaagacacatacgacgcactccatatgcaggctctcccacctaga

SEQ ID NO: 56 - DNA, 1893 bp, synthetic construct
  source 1..1893: mol_type = other DNA; note = chimeric antigen receptor
atggcccttccagtgaccgccctgctgctgccactggctctgctgctgcacgccgctagacctcaggtgcagctggtggaaagcgggggaggcctggttcagcccggcggcagcctgagactgagctgcgccgctagcggcagaacattcagcaactacaacatgggctggttcagacaagcccctggccagggcctggaattcgtggccgctatcgactggtccggcggcagcccttactacgccgcctccgtgcggggcagattcaccatctctcgggataatagcaagaacaccctctacctgcagatgaatagcctgagagccgaggataccgccgtgtactactgtgccgctcctctgtcttacggcagcacctggctggcagattactggggccagggcaccctggtgacagtgtccagcggcggaggaggcagcggcggaggcggaagcggcggtggtggctctggaggcggcggctccggcggtggcggcagtgatatccagatgacccagaccacttccagcctgtctgcctccctgggcgacagggtgactatcagctgccgcgccagccaggatatttcaaaatacctgaattggtaccagcagaagcccgacggcacagtgaagctgctgatctaccacaccagtcgcctgcacagcggcgtgcccagcaggttcagcggcagcggatccggcacagactacagcctgaccatcagcaacctggagcaggaggatatcgcaacttatttttgccagcagggcaatacactgccttacaccttcggcggcggcaccaagctggaaatcaccggcagcacaagtggctccggcaaaccaggcagcggagagggcagcacaaagggcgaggtgaaactgcaggagagcggccccggcctggtggcccccagccagtctctgagcgtgacctgcaccgtgtccggcgtgtccctgcctgactacggggtgagctggatcaggcagccccccaggaaaggcttggaatggctgggcgtgatctggggcagcgagacaacctattataactctgccctgaagagcagactgaccatcatcaaagacaatagcaaaagccaggtgttcctgaagatgaattcactgcagactgacgatactgccatctattattgtgccaaacactactactatggcggatcctatgccatggattactggggccagggcacctcagtgaccgtgtcctcgattgaagtgatgtatccacccccttacctggacaacgagaaatcaaacggcactattatccacgtgaagggaaagcacctgtgcccctcccctctgtttcccggcccaagtaagcccttttgggtgctggtggtggtcgggggcgtgctggcctgttattccctgctggtcacagtggctttcatcatcttctgggtgcgcagcaagaggtccagactgctgcactctgactacatgaacatgactcccaggaggccaggccctactagaaaacactaccagccctacgctcctcctagagacttcgccgcctacaggtccagggtcaagttttccagaagcgctgacgctcccgcttaccagcagggccaaaatcagctctataacgaactgaatctcggcaggcgcgaggaatatgacgtgctggataagaggcggggacgcgaccctgaaatgggaggaaagcctcggcggaaaaacccacaagaaggactttacaacgaactccaaaaggataagatggctgaagcctactctgagattggcatgaaaggagaacgtcggagaggaaaaggccacgacggactctatcagggactgtctacagccacaaaagacacatacgacgcactccatatgcaggctctcccacctaga

SEQ ID NO: 57 - protein, 888 aa, synthetic construct
  source 1..888: note = chimeric antigen receptor
MALPVTALLLPLALLLHAARPQVQLVESGGGLVQPGGSLRLSCAASGRTFSNYNMGWFRQAPGQGLEFVAAIDWSGGSPYYAASVRGRFTISRDNSKNTLYLQMNSLRAEDTAVYYCAAPLSYGSTWLADYWGQGTLVTVSSGGGGSGGGGSGGGGSGGGGSGGGGSDIQMTQTTSSLSASLGDRVTISCRASQDISKYLNWYQQKPDGTVKLLIYHTSRLHSGVPSRFSGSGSGTDYSLTISNLEQEDIATYFCQQGNTLPYTFGGGTKLEITGSTSGSGKPGSGEGSTKGEVKLQESGPGLVAPSQSLSVTCTVSGVSLPDYGVSWIRQPPRKGLEWLGVIWGSETTYYNSALKSRLTIIKDNSKSQVFLKMNSLQTDDTAIYYCAKHYYYGGSYAMDYWGQGTSVTVSSIEVMYPPPYLDNEKSNGTIIHVKGKHLCPSPLFPGPSKPFWVLVVVGGVLACYSLLVTVAFIIFWVKRGRKKLLYIFKQPFMRPVQTTQEEDGCSCRFPEEEEGGCELRVKFSRSADAPAYQQGQNQLYNELNLGRREEYDVLDKRRGRDPEMGGKPRRKNPQEGLYNELQKDKMAEAYSEIGMKGERRRGKGHDGLYQGLSTATKDTYDALHMQALPPRRAKRSGSGEGRGSLLTCGDVEENPGPMDMRVPAQLLGLLLLWLRGARCEFKPLPEVTDEYAAAESKYGPPCPPCPMFWVLVVVGGVLACYSLLVTVAFIIFWVRSKRSRLLHSDYMNMTPRRPGPTRKHYQPYAPPRDFAAYRSRVKFSRSADAPAYQQGQNQLYNELNLGRREEYDVLDKRRGRDPEMGGKPRRKNPQEGLYNELQKDKMAEAYSEIGMKGERRRGKGHDGLYQGLSTATKDTYDALHMQALPPR

SEQ ID NO: 58 - protein, 887 aa, synthetic construct
  source 1..887: note = chimeric antigen receptor
MDMRVPAQLLGLLLLWLRGARCEFKPLPEVTDEYAAAESKYGPPCPPCPDIYIWAPLAGTCGVLLLSLVITLYCRSKRSRLLHSDYMNMTPRRPGPTRKHYQPYAPPRDFAAYRSRVKFSRSADAPAYQQGQNQLYNELNLGRREEYDVLDKRRGRDPEMGGKPRRKNPQEGLYNELQKDKMAEAYSEIGMKGERRRGKGHDGLYQGLSTATKDTYDALHMQALPPRGSGSSGEGRGSLLTCGDVEENPGPPVATMALPVTALLLPLALLLHAARPQVQLVESGGGLVQPGGSLRLSCAASGRTFSNYNMGWFRQAPGQGLEFVAAIDWSGGSPYYAASVRGRFTISRDNSKNTLYLQMNSLRAEDTAVYYCAAPLSYGSTWLADYWGQGTLVTVSSGGGGSGGGGSGGGGSGGGGSGGGGSDIQMTQTTSSLSASLGDRVTISCRASQDISKYLNWYQQKPDGTVKLLIYHTSRLHSGVPSRFSGSGSGTDYSLTISNLEQEDIATYFCQQGNTLPYTFGGGTKLEITGSTSGSGKPGSGEGSTKGEVKLQESGPGLVAPSQSLSVTCTVSGVSLPDYGVSWIRQPPRKGLEWLGVIWGSETTYYNSALKSRLTIIKDNSKSQVFLKMNSLQTDDTAIYYCAKHYYYGGSYAMDYWGQGTSVTVSSIEVMYPPPYLDNEKSNGTIIHVKGKHLCPSPLFPGPSKPFWVLVVVGGVLACYSLLVTVAFIIFWVKRGRKKLLYIFKQPFMRPVQTTQEEDGCSCRFPEEEEGGCELRVKFSRSADAPAYQQGQNQLYNELNLGRREEYDVLDKRRGRDPEMGGKPRRKNPQEGLYNELQKDKMAEAYSEIGMKGERRRGKGHDGLYQGLSTATKDTYDALHMQALPPR

SEQ ID NO: 59 - protein, 888 aa, synthetic construct
  source 1..888: note = chimeric antigen receptor
MALPVTALLLPLALLLHAARPQVQLVESGGGLVQPGGSLRLSCAASGRTFSNYNMGWFRQAPGQGLEFVAAIDWSGGSPYYAASVRGRFTISRDNSKNTLYLQMNSLRAEDTAVYYCAAPLSYGSTWLADYWGQGTLVTVSSGGGGSGGGGSGGGGSGGGGSGGGGSDIQMTQTTSSLSASLGDRVTISCRASQDISKYLNWYQQKPDGTVKLLIYHTSRLHSGVPSRFSGSGSGTDYSLTISNLEQEDIATYFCQQGNTLPYTFGGGTKLEITGSTSGSGKPGSGEGSTKGEVKLQESGPGLVAPSQSLSVTCTVSGVSLPDYGVSWIRQPPRKGLEWLGVIWGSETTYYNSALKSRLTIIKDNSKSQVFLKMNSLQTDDTAIYYCAKHYYYGGSYAMDYWGQGTSVTVSSIEVMYPPPYLDNEKSNGTIIHVKGKHLCPSPLFPGPSKPFWVLVVVGGVLACYSLLVTVAFIIFWVRSKRSRLLHSDYMNMTPRRPGPTRKHYQPYAPPRDFAAYRSRVKFSRSADAPAYQQGQNQLYNELNLGRREEYDVLDKRRGRDPEMGGKPRRKNPQEGLYNELQKDKMAEAYSEIGMKGERRRGKGHDGLYQGLSTATKDTYDALHMQALPPRRAKRSGSGEGRGSLLTCGDVEENPGPMDMRVPAQLLGLLLLWLRGARCEFKPLPEVTDEYAAAESKYGPPCPPCPMFWVLVVVGGVLACYSLLVTVAFIIFWVKRGRKKLLYIFKQPFMRPVQTTQEEDGCSCRFPEEEEGGCELRVKFSRSADAPAYQQGQNQLYNELNLGRREEYDVLDKRRGRDPEMGGKPRRKNPQEGLYNELQKDKMAEAYSEIGMKGERRRGKGHDGLYQGLSTATKDTYDALHMQALPPR

SEQ ID NO: 60 - protein, 887 aa, synthetic construct
  source 1..887: note = chimeric antigen receptor
MDMRVPAQLLGLLLLWLRGARCEFKPLPEVTDEYAAAESKYGPPCPPCPDIYIWAPLAGTCGVLLLSLVITLYCKRGRKKLLYIFKQPFMRPVQTTQEEDGCSCRFPEEEEGGCELRVKFSRSADAPAYQQGQNQLYNELNLGRREEYDVLDKRRGRDPEMGGKPRRKNPQEGLYNELQKDKMAEAYSEIGMKGERRRGKGHDGLYQGLSTATKDTYDALHMQALPPRGSGSSGEGRGSLLTCGDVEENPGPPVATMALPVTALLLPLALLLHAARPQVQLVESGGGLVQPGGSLRLSCAASGRTFSNYNMGWFRQAPGQGLEFVAAIDWSGGSPYYAASVRGRFTISRDNSKNTLYLQMNSLRAEDTAVYYCAAPLSYGSTWLADYWGQGTLVTVSSGGGGSGGGGSGGGGSGGGGSGGGGSDIQMTQTTSSLSASLGDRVTISCRASQDISKYLNWYQQKPDGTVKLLIYHTSRLHSGVPSRFSGSGSGTDYSLTISNLEQEDIATYFCQQGNTLPYTFGGGTKLEITGSTSGSGKPGSGEGSTKGEVKLQESGPGLVAPSQSLSVTCTVSGVSLPDYGVSWIRQPPRKGLEWLGVIWGSETTYYNSALKSRLTIIKDNSKSQVFLKMNSLQTDDTAIYYCAKHYYYGGSYAMDYWGQGTSVTVSSIEVMYPPPYLDNEKSNGTIIHVKGKHLCPSPLFPGPSKPFWVLVVVGGVLACYSLLVTVAFIIFWVRSKRSRLLHSDYMNMTPRRPGPTRKHYQPYAPPRDFAAYRSRVKFSRSADAPAYQQGQNQLYNELNLGRREEYDVLDKRRGRDPEMGGKPRRKNPQEGLYNELQKDKMAEAYSEIGMKGERRRGKGHDGLYQGLSTATKDTYDALHMQALPPR

SEQ ID NO: 61 - protein, 914 aa, synthetic construct
  source 1..914: note = chimeric antigen receptor
MALPVTALLLPLALLLHAARPQVQLVESGGGLVQPGGSLRLSCAASGRTFSNYNMGWFRQAPGQGLEFVAAIDWSGGSPYYAASVRGRFTISRDNSKNTLYLQMNSLRAEDTAVYYCAAPLSYGSTWLADYWGQGTLVTVSSGGGGSGGGGSGGGGSGGGGSGGGGSDIQMTQTTSSLSASLGDRVTISCRASQDISKYLNWYQQKPDGTVKLLIYHTSRLHSGVPSRFSGSGSGTDYSLTISNLEQEDIATYFCQQGNTLPYTFGGGTKLEITGSTSGSGKPGSGEGSTKGEVKLQESGPGLVAPSQSLSVTCTVSGVSLPDYGVSWIRQPPRKGLEWLGVIWGSETTYYNSALKSRLTIIKDNSKSQVFLKMNSLQTDDTAIYYCAKHYYYGGSYAMDYWGQGTSVTVSSIEVMYPPPYLDNEKSNGTIIHVKGKHLCPSPLFPGPSKPFWVLVVVGGVLACYSLLVTVAFIIFWVRSKRSRLLHSDYMNMTPRRPGPTRKHYQPYAPPRDFAAYRSRVKFSRSADAPAYQQGQNQLYNELNLGRREEYDVLDKRRGRDPEMGGKPRRKNPQEGLYNELQKDKMAEAYSEIGMKGERRRGKGHDGLYQGLSTATKDTYDALHMQALPPRRAKRSGSGEGRGSLLTCGDVEENPGPMDMRVPAQLLGLLLLWLRGARCEFKPLPEVTDEYAAAIEVMYPPPYLDNEKSNGTIIHVKGKHLCPSPLFPGPSKPFWVLVVVGGVLACYSLLVTVAFIIFWVKRGRKKLLYIFKQPFMRPVQTTQEEDGCSCRFPEEEEGGCELRVKFSRSADAPAYQQGQNQLYNELNLGRREEYDVLDKRRGRDPEMGGKPRRKNPQEGLYNELQKDKMAEAYSEIGMKGERRRGKGHDGLYQGLSTATKDTYDALHMQALPPR

SEQ ID NO: 62 - protein, 915 aa, synthetic construct
  source 1..915: note = chimeric antigen receptor
MALPVTALLLPLALLLHAARPQVQLVESGGGLVQPGGSLRLSCAASGRTFSNYNMGWFRQAPGQGLEFVAAIDWSGGSPYYAASVRGRFTISRDNSKNTLYLQMNSLRAEDTAVYYCAAPLSYGSTWLADYWGQGTLVTVSSGGGGSGGGGSGGGGSGGGGSGGGGSDIQMTQTTSSLSASLGDRVTISCRASQDISKYLNWYQQKPDGTVKLLIYHTSRLHSGVPSRFSGSGSGTDYSLTISNLEQEDIATYFCQQGNTLPYTFGGGTKLEITGSTSGSGKPGSGEGSTKGEVKLQESGPGLVAPSQSLSVTCTVSGVSLPDYGVSWIRQPPRKGLEWLGVIWGSETTYYNSALKSRLTIIKDNSKSQVFLKMNSLQTDDTAIYYCAKHYYYGGSYAMDYWGQGTSVTVSSAAAIEVMYPPPYLDNEKSNGTIIHVKGKHLCPSPLFPGPSKPFWVLVVVGGVLACYSLLVTVAFIIFWVRSKRSRLLHSDYMNMTPRRPGPTRKHYQPYAPPRDFAAYRSRVKFSRSADAPAYQQGQNQLYNELNLGRREEYDVLDKRRGRDPEMGGKPRRKNPQEGLYNELQKDKMAEAYSEIGMKGERRRGKGHDGLYQGLSTATKDTYDALHMQALPPRRAKRSGSGEGRGSLLTCGDVEENPGPMDMRVPAQLLGLLLLWLRGARCEFKPLPEVTDEYDIEVMYPPPYLDNEKSNGTIIHVKGKHLCPSPLFPGPSKPFWVLVVVGGVLACYSLLVTVAFIIFWVKRGRKKLLYIFKQPFMRPVQTTQEEDGCSCRFPEEEEGGCELRVKFSRSADAPAYQQGQNQLYNELNLGRREEYDVLDKRRGRDPEMGGKPRRKNPQEGLYNELQKDKMAEAYSEIGMKGERRRGKGHDGLYQGLSTATKDTYDALHMQALPPR

SEQ ID NO: 63 - protein, 884 aa, synthetic construct
  source 1..884: note = chimeric antigen receptor
MALPVTALLLPLALLLHAARPQVQLVESGGGLVQPGGSLRLSCAASGRTFSNYNMGWFRQAPGQGLEFVAAIDWSGGSPYYAASVRGRFTISRDNSKNTLYLQMNSLRAEDTAVYYCAAPLSYGSTWLADYWGQGTLVTVSSGGGGSGGGGSGGGGSGGGGSGGGGSDIQMTQTTSSLSASLGDRVTISCRASQDISKYLNWYQQKPDGTVKLLIYHTSRLHSGVPSRFSGSGSGTDYSLTISNLEQEDIATYFCQQGNTLPYTFGGGTKLEITGSTSGSGKPGSGEGSTKGEVKLQESGPGLVAPSQSLSVTCTVSGVSLPDYGVSWIRQPPRKGLEWLGVIWGSETTYYNSALKSRLTIIKDNSKSQVFLKMNSLQTDDTAIYYCAKHYYYGGSYAMDYWGQGTSVTVSSIEVMYPPPYLDNEKSNGTIIHVKGKHLCPSPLFPGPSKPFWVLVVVGGVLACYSLLVTVAFIIFWVRSKRSRLLHSDYMNMTPRRPGPTRKHYQPYAPPRDFAAYRSRVKFSRSADAPAYQQGQNQLYNELNLGRREEYDVLDKRRGRDPEMGGKPRRKNPQEGLYNELQKDKMAEAYSEIGMKGERRRGKGHDGLYQGLSTATKDTYDALHMQALPPRRAKRSGSGEGRGSLLTCGDVEENPGPMDMRVPAQLLGLLLLWLRGARCEFKPLPEVTDEYAAAESKYGPPCPPCPIYIWAPLAGTCGVLLLSLVITLYCKRGRKKLLYIFKQPFMRPVQTTQEEDGCSCRFPEEEEGGCELRVKFSRSADAPAYQQGQNQLYNELNLGRREEYDVLDKRRGRDPEMGGKPRRKNPQEGLYNELQKDKMAEAYSEIGMKGERRRGKGHDGLYQGLSTATKDTYDALHMQALPPR

SEQ ID NO: 64 - DNA, 2667 bp, synthetic construct
  source 1..2667: mol_type = other DNA; note = chimeric antigen receptor
atggcccttccagtgaccgccctgctgctgccactggctctgctgctgcacgccgctagacctcaggtgcagctggtggaaagcggcgggggcctggtgcagcctggcggcagcctgagactgtcttgcgccgctagcggaagaacttttagcaactacaacatgggctggtttagacaggcccccggccagggcctggagttcgtggctgccatcgactggagcggcggaagcccctattacgccgcctccgtgcggggcagattcaccatcagccgggacaattctaagaataccctgtatctgcaaatgaacagcctgagagccgaagatacagccgtgtactactgcgccgcccctctgagctacggaagcacatggctggccgactactggggacaaggaaccctggtaaccgtctcaagcggcggtggaggatcaggaggtggtggttcaggaggtggaggttctgggggaggcggatctgggggaggaggcagcgacatccagatgacacagacaacctccagcctgagcgccagcctgggcgacagagtgaccatcagctgtagagcctctcaggacatcagcaagtacctgaactggtatcagcagaaacctgatggcaccgtgaagctgctgatctaccacacatctaggctgcactctggagtccccagccggtttagcggaagcgggtcaggcacagactatagcctgaccatctccaatctggaacaggaggacatcgccacctacttctgccagcagggcaacaccctgccttatacattcggtggcggcaccaagctggaaatcaccggcagcacctctggctctggcaagcccggaagcggcgagggctccaccaagggagaggtgaagctgcaggagtccggacctgggctggtggctccaagccagagcctgagcgtgacctgcaccgtgtccggagtgagcctgcctgattacggcgtgtcttggatcagacagcctcctagaaagggactggaatggctgggcgtgatctggggtagcgagacaacatactacaacagcgccctgaagagcagactgacaatcatcaaggacaacagcaaaagccaggtgttcctaaaaatgaactccctgcagaccgacgacaccgccatctactactgtgcgaaacactactactacggcggctcctacgccatggactattggggccagggcaccagcgtgacagtgagcagcatcgaggtgatgtacccccctccttacctggacaacgagaagtccaacggcaccattatccacgtgaaaggcaagcacctgtgccccagccctctgttccccggcccttctaaaccgttctgggttctggtggtcgtgggcggcgtactggcttgctactctctgctggtcacagtggctttcatcatcttctgggtgaaaagaggcagaaagaaactgctgtacatctttaagcagccattcatgcggccagtgcagaccacccaggaggaggacggctgctcttgtcgctttcccgaggaggaggagggcggatgtgagctgagggtgaagtttagcagatccgctgatgcccctgcctatcagcagggacagaaccagctgtacaacgagctgaacctggggagaagagaagagtacgatgtgctggacaagcggagaggcagagatcctgagatgggcggcaagcccagacggaagaatcctcaagagggcctgtacaatgaactgcagaaagacaagatggccgaggcctacagcgagatcggaatgaagggcgagcgcagaagaggcaagggacacgatggactgtaccagggcctgagcaccgccaccaaggatacctatgatgccctgcacatgcaggccctgcctccaagaagagcaaagagatccggaagcggcgaaggcagaggatcactgcttacatgcggcgacgtggaagagaaccctggacctatggacatgagagtgccagctcagctgctgggcctgctgctgctgtggctgagaggcgccagatgcgagttcaagcctctgcctgaagtgaccgacgagtacgccgccgctgagtctaagtacggccctccttgtcctccttgccctatgttttgggtgctggttgtggttggaggcgtgctcgcttgttactccctcctggtgacagtcgcttttatcattttttgggtgcgcagcaagaggtccagactgctgcactctgactacatgaacatgactcccaggaggccaggccctactagaaaacactaccagccctacgctcctcctagagacttcgccgcctacaggtccagggtcaagttttccagaagcgctgacgctcccgcttaccagcagggccaaaatcagctctataacgaactgaatctcggcaggcgcgaggaatatgacgtgctggataagaggcggggacgcgaccctgaaatgggaggaaagcctcggcggaaaaacccacaagaaggactttacaacgaactccaaaaggataagatggctgaagcctactctgagattggcatgaaaggagaacgtcggagaggaaaaggccacgacggactctatcagggactgtctacagccacaaaagacacatacgacgcactccatatgcaggctctcccacctagataa

SEQ ID NO: 65 - DNA, 2664 bp, synthetic construct
  source 1..2664: mol_type = other DNA; note = chimeric antigen receptor
atggatatgagggtgccagcccagctgctgggcctgctgctgctgtggctgagaggagccaggtgtgaatttaagcccctgcctgaggtgactgacgagtacgccgcagctgagtccaagtacggcccaccctgcccaccctgcccagacatctacatttgggcccctctggccggaacatgcggagtgctgcttctgtcccttgtaatcaccctttattgtcgatccaagagatcacgactgctgcattctgattacatgaatatgactcctagacggccagggcccacaaggaagcactaccagccttatgcccctcctagagatttcgccgcctatagaagtagggtgaagtttagcagatccgctgatgcccctgcctatcagcagggacagaaccagctgtacaacgagctgaacctggggagaagagaagagtacgatgtgctggacaagcggagaggcagagatcctgagatgggcggcaagcccagacggaagaatcctcaagagggcctgtacaatgaactgcagaaagacaagatggccgaggcctacagcgagatcggaatgaagggcgagcgcagaagaggcaagggacacgatggactgtaccagggcctgagcaccgccaccaaggatacctatgatgccctgcacatgcaggcactgcctccaagaggatctggctcgagcggcgaaggcagaggatcactgcttacatgcggcgacgtggaagagaaccctggacctcctgtggccaccatggccctgccagtgaccgccctgctgctgcccctggcactgctgctgcacgcagccagaccccaagtgcagctggtggagtcaggcggcgggctagtgcagccaggaggctccctgagactgtcttgcgctgcaagcggcagaaccttctcaaactacaatatggggtggttcaggcaggcccccgggcagggcctggagttcgtggccgctatcgactggagtgggggctccccctactatgcagctagcgtgagaggcagatttaccatctccagagacaactccaagaacactctgtacctccagatgaatagtctgagagccgaagatacagccgtgtactactgtgccgcccccctgagctacggcagcacctggctggctgattactggggtcagggaacactggttacagtgtcatccggaggaggtggtagtggaggcggaggcagtggtggaggcggtagcgggggaggcggatctgggggaggaggcagcgacatccagatgacccagaccacctcctctctgagcgcttcactcggagaccgggtgacaatcagctgtagagcctcccaggatatctctaagtatctgaactggtaccagcagaagccagatggcacagtgaagctgctgatctatcataccagcaggctgcactccggagtgccttccaggttttccggcagcggatccggcaccgattatagcctgaccatctccaatctggagcaggaggacatagcaacctacttttgccagcagggcaataccctgccctacacctttgggggaggaaccaaactcgaaatcaccggctctacttctggaagcggcaagcccggatcaggcgaaggctcaaccaagggcgaggtgaaactgcaggagagcggcccaggactggtcgccccatcacagtccctgtcagtgacctgcaccgttagcggggtgtccctgcctgactacggggtgagctggatcaggcagcctcctcggaagggcctggagtggctgggggtgatctggggctccgagaccacctattataactccgccctgaagtcccggctgaccatcattaaagataacagcaagagccaggtgttcctgaagatgaactcactgcagacagacgacaccgctatctattattgcgccaagcattactactacggcggatcatacgccatggactattggggccagggcacttctgtgaccgtgtcttctatcgaggtgatgtaccccccaccatatctggataacgagaaatccaatggcaccatcattcacgtgaagggcaagcacctgtgtccatctcctctgttccctggcccaagcaagcccttctgggtgctggtggtcgtggggggcgtgctggcctgctactctctgctggtgactgtggcattcatcatcttctgggtgaagcggggcaggaagaaactgctgtacatcttcaagcagccattcatgcggcccgtgcagaccacccaggaagaggatgggtgctcatgccggttccctgaggaggaggagggggggtgcgagctgagggtcaagttttccagaagcgctgacgctcccgcttaccagcagggccaaaatcagctctataacgaactgaatctcggcaggcgcgaggaatatgacgtgctggataagaggcggggacgcgaccctgaaatgggaggaaagcctcggcggaaaaacccacaagaaggactttacaacgaactccaaaaggataagatggctgaagcctactctgagattggcatgaaaggagaacgtcggagaggaaaaggccacgacggactctatcagggactgtctacagccacaaaagacacatacgacgcactccatatgcaggctctcccacctagataa

SEQ ID NO: 66 - DNA, 2667 bp, synthetic construct
  source 1..2667: mol_type = other DNA; note = chimeric antigen receptor
atggccctgccagtgaccgccctgctgctgcccctggcactgctgctgcacgcagccagaccccaagtgcagctggtggagtcaggcggcgggctagtgcagccaggaggctccctgagactgtcttgcgctgcaagcggcagaaccttctcaaactacaatatggggtggttcaggcaggcccccgggcagggcctggagttcgtggccgctatcgactggagtgggggctccccctactatgcagctagcgtgagaggcagatttaccatctccagagacaactccaagaacactctgtacctccagatgaatagtctgagagccgaagatacagccgtgtactactgtgccgcccccctgagctacggcagcacctggctggctgattactggggacagggtacactggttacagtatcatctggcggtggaggatcaggaggtggtggttcaggaggtggaggttctgggggaggcggatctgggggaggaggcagcgacatccagatgacccagaccacctcctctctgagcgcttcactcggagaccgggtgacaatcagctgtagagcctcccaggatatctctaagtatctgaactggtaccagcagaagccagatggcacagtgaagctgctgatctatcataccagcaggctgcactccggagtgccttccaggttttccggcagcggatccggcaccgattatagcctgaccatctccaatctggagcaggaggacatagcaacctacttttgccagcagggcaataccctgccctacacctttgggggaggaaccaaactcgaaatcaccggctctacttctggaagcggcaagcccggatcaggcgaaggctcaaccaagggcgaggtgaaactgcaggagagcggcccaggactggtcgccccatcacagtccctgtcagtgacctgcaccgttagcggggtgtccctgcctgactacggggtgagctggatcaggcagcctcctcggaagggcctggagtggctgggggtgatctggggctccgagaccacctattataactccgccctgaagtcccggctgaccatcattaaagataacagcaagagccaggtgttcctgaagatgaactcactgcagacagacgacaccgctatctattattgcgccaagcattactactacggcggatcatacgccatggactattggggccagggcacttctgtgaccgtgtcttctatcgaggtgatgtaccccccaccatatctggataacgagaaatccaatggcaccatcattcacgtgaagggcaagcacctgtgtccatctcctctgttccctggcccaagcaagcccttctgggtgctggtggtcgtggggggcgtgctggcctgctactctctgctggtgactgtggcattcatcatcttctgggtgagatccaaaaggtctcgcctgctgcacagcgactatatgaatatgacccctcgcaggcctggccctacacgcaagcactatcagccttacgccccccctcgggactttgctgcgtatcggagtagggtgaagtttagcagatccgctgatgcccctgcctatcagcagggacagaaccagctgtacaacgagctgaacctggggagaagagaagagtacgatgtgctggacaagcggagaggcagagatcctgagatgggcggcaagcccagacggaagaatcctcaagagggcctgtacaatgaactgcagaaagacaagatggccgaggcctacagcgagatcggaatgaagggcgagcgcagaagaggcaagggacacgatggactgtaccagggcctgagcaccgccaccaaggatacctatgatgccctgcacatgcaggccctgcctccaagaagagcaaagagatccggaagcggcgaaggcagaggatcactgcttacatgcggcgacgtggaagagaaccctggacctatggacatgagagtgccagctcagctgctgggcctgctgctgctgtggctgagaggcgccagatgcgagttcaagcctctgcctgaagtgaccgacgagtacgccgccgctgagtctaagtacggccctccttgtcctccttgccctatgttttgggtcctggttgtggttggaggcgtgctcgcttgttactccctcctggtgacagtcgcttttatcattttttgggtgaagaggggccgcaagaagctgctgtatatctttaagcagccatttatgcggcccgtgcagaccacccaagaagaggacggatgtagctgcagatttcctgaggaagaagagggcggctgtgaactgagggtcaagttttccagaagcgctgacgctcccgcttaccagcagggccaaaatcagctctataacgaactgaatctcggcaggcgcgaggaatatgacgtgctggataagaggcggggacgcgaccctgaaatgggaggaaagcctcggcggaaaaacccacaagaaggactttacaacgaactccaaaaggataagatggctgaagcctactctgagattggcatgaaaggagaacgtcggagaggaaaaggccacgacggactctatcagggactgtctacagccacaaaagacacatacgacgcactccatatgcaggctctcccacctagataa

SEQ ID NO: 67 - DNA, 2664 bp, synthetic construct
  source 1..2664: mol_type = other DNA; note = chimeric antigen receptor
atggatatgagagtgccagcccagctgctgggcctgctgctgctgtggctgagaggcgccagatgcgagttcaagcctctgccagaggtgactgatgagtacgccgctgcagaatcaaagtacggccctccttgtccaccctgtccagacatctacatttgggcccccctggccgggacatgcggcgtgctcctgctgtctctggtgatcaccctgtactgtaaaagaggcagaaagaaactgctgtacatctttaagcagccattcatgcggccagtgcagaccacccaggaggaggacggctgctcttgtcgctttcccgaggaggaggagggcggatgtgagctgagggtgaagtttagcagatccgctgatgcccctgcctatcagcagggacagaaccagctgtacaacgagctgaacctggggagaagagaagagtacgatgtgctggacaagcggagaggcagagatcctgagatgggcggcaagcccagacggaagaatcctcaagagggcctgtacaatgaactgcagaaagacaagatggccgaggcctacagcgagatcggaatgaagggcgagcgcagaagaggcaagggacacgatggactgtaccagggcctgagcaccgccaccaaggatacctatgatgccctgcacatgcaggcactgcctccaagaggatctggctcgagcggcgaaggcagaggatcactgcttacatgcggcgacgtggaagagaaccctggacctcctgtggccaccatggccctgccagtgaccgccctgctgctgcccctggcactgctgctgcacgcagccagaccccaagtgcagctggtggagtcaggcggcgggctagtgcagccaggaggctccctgagactgtcttgcgctgcaagcggcagaaccttctcaaactacaatatggggtggttcaggcaggcccccgggcagggcctggagttcgtggccgctatcgactggagtgggggctccccctactatgcagctagcgtgagaggcagatttaccatctccagagacaactccaagaacactctgtacctccagatgaatagtctgagagccgaagatacagccgtgtactactgtgccgcccccctgagctacggcagcacctggctggctgattactggggacagggtacactggttacagtatcatctggcggtggaggatcaggaggtggtggttcaggaggtggaggttctgggggaggcggatctgggggaggaggcagcgacatccagatgacccagaccacctcctctctgagcgcttcactcggagaccgggtgacaatcagctgtagagcctcccaggatatctctaagtatctgaactggtaccagcagaagccagatggcacagtgaagctgctgatctatcataccagcaggctgcactccggagtgccttccaggttttccggcagcggatccggcaccgattatagcctgaccatctccaatctggagcaggaggacatagcaacctacttttgccagcagggcaataccctgccctacacctttgggggaggaaccaaactcgaaatcaccggctctacttctggaagcggcaagcccggatcaggcgaaggctcaaccaagggcgaggtgaaactgcaggagagcggcccaggactggtcgccccatcacagtccctgtcagtgacctgcaccgttagcggggtgtccctgcctgactacggggtgagctggatcaggcagcctcctcggaagggcctggagtggctgggggtgatctggggctccgagaccacctattataactccgccctgaagtcccggctgaccatcattaaagataacagcaagagccaggtgttcctgaagatgaactcactgcagacagacgacaccgctatctattattgcgccaagcattactactacggcggatcatacgccatggactattggggccagggcacttctgtgaccgtgtcttctatcgaggtgatgtaccccccaccatatctggataacgagaaatccaatggcaccatcattcacgtgaagggcaagcacctgtgtccatctcctctgttccctggcccaagcaagcccttctgggtgctggtggtcgtggggggcgtgctggcctgctactctctgctggtgactgtggcattcatcatcttctgggtgagatccaaaaggtctcgcctgctgcacagcgactatatgaatatgacccctcgcaggcctggccctacacgcaagcactatcagccttacgccccccctcgggactttgctgcgtatcggagtagggtcaagttttccagaagcgctgacgctcccgcttaccagcagggccaaaatcagctctataacgaactgaatctcggcaggcgcgaggaatatgacgtgctggataagaggcggggacgcgaccctgaaatgggaggaaagcctcggcggaaaaacccacaagaaggactttacaacgaactccaaaaggataagatggctgaagcctactctgagattggcatgaaaggagaacgtcggagaggaaaaggccacgacggactctatcagggactgtctacagccacaaaagacacatacgacgcactccatatgcaggctctcccacctagataa

SEQ ID NO: 68 - DNA, 2745 bp, synthetic construct
  source 1..2745: mol_type = other DNA; note = chimeric antigen receptor
atggccctgccagtgaccgccctgctgctgcccctggcactgctgctgcacgcagccagaccccaagtgcagctggtggagtcaggcggcgggctagtgcagccaggaggctccctgagactgtcttgcgctgcaagcggcagaaccttctcaaactacaatatggggtggttcaggcaggcccccgggcagggcctggagttcgtggccgctatcgactggagtgggggctccccctactatgcagctagcgtgagaggcagatttaccatctccagagacaactccaagaacactctgtacctccagatgaatagtctgagagccgaagatacagccgtgtactactgtgccgcccccctgagctacggcagcacctggctggctgattactggggacagggtacactggttacagtatcatctggcggtggaggatcaggaggtggtggttcaggaggtggaggttctgggggaggcggatctgggggaggaggcagcgacatccagatgacccagaccacctcctctctgagcgcttcactcggagaccgggtgacaatcagctgtagagcctcccaggatatctctaagtatctgaactggtaccagcagaagccagatggcacagtgaagctgctgatctatcataccagcaggctgcactccggagtgccttccaggttttccggcagcggatccggcaccgattatagcctgaccatctccaatctggagcaggaggacatagcaacctacttttgccagcagggcaataccctgccctacacctttgggggaggaaccaaactcgaaatcaccggctctacttctggaagcggcaagcccggatcaggcgaaggctcaaccaagggcgaggtgaaactgcaggagagcggcccaggactggtcgccccatcacagtccctgtcagtgacctgcaccgttagcggggtgtccctgcctgactacggggtgagctggatcaggcagcctcctcggaagggcctggagtggctgggggtgatctggggctccgagaccacctattataactccgccctgaagtcccggctgaccatcattaaagataacagcaagagccaggtgttcctgaagatgaactcactgcagacagacgacaccgctatctattattgcgccaagcattactactacggcggatcatacgccatggactattggggccagggcacttctgtgaccgtgtcttctatcgaggtgatgtaccccccaccatatctggataacgagaaatccaatggcaccatcattcacgtgaagggcaagcacctgtgtccatctcctctgttccctggcccaagcaagcccttctgggtgctggtggtcgtggggggcgtgctggcctgctactctctgctggtgactgtggcattcatcatcttctgggtgagatccaaaaggtctcgcctgctgcacagcgactatatgaatatgacccctcgcaggcctggccctacacgcaagcactatcagccttacgccccccctcgggactttgctgcgtatcggagtagggtgaagtttagcagatccgctgatgcccctgcctatcagcagggacagaaccagctgtacaacgagctgaacctggggagaagagaagagtacgatgtgctggacaagcggagaggcagagatcctgagatgggcggcaagcccagacggaagaatcctcaagagggcctgtacaatgaactgcagaaagacaagatggccgaggcctacagcgagatcggaatgaagggcgagcgcagaagaggcaagggacacgatggactgtaccagggcctgagcaccgccaccaaggatacctatgatgccctgcacatgcaggccctgcctccaagaagagcaaagagatccggaagcggcgaaggcagaggatcactgcttacatgcggcgacgtggaagagaaccctggacctatggacatgagagtgccagctcagctgctgggcctgctgctgctgtggctgagaggcgccagatgcgagttcaagcctctgcctgaagtgaccgacgagtacgccgccgctattgaagtcatgtatccacctccctatctggacaatgaaaagtctaatggcacaatcatccacgtcaagggaaaacacctgtgccctagccccctgtttcctggcccctctaaacccttttgggtcctggttgtggttggaggcgtgctcgcttgttactccctcctggtgacagtcgcttttatcattttttgggtgaagaggggccgcaagaagctgctgtatatctttaagcagccatttatgcggcccgtgcagaccacccaagaagaggacggatgtagctgcagatttcctgaggaagaagagggcggctgtgaactgagggtcaagttttccagaagcgctgacgctcccgcttaccagcagggccaaaatcagctctataacgaactgaatctcggcaggcgcgaggaatatgacgtgctggataagaggcggggacgcgaccctgaaatgggaggaaagcctcggcggaaaaacccacaagaaggactttacaacgaactccaaaaggataagatggctgaagcctactctgagattggcatgaaaggagaacgtcggagaggaaaaggccacgacggactctatcagggactgtctacagccacaaaagacacatacgacgcactccatatgcaggctctcccacctagataa

SEQ ID NO: 69 - DNA, 2748 bp, synthetic construct
  source 1..2748: mol_type = other DNA; note = chimeric antigen receptor
atggcccttccagtgaccgccctgctgctgccactggctctgctgctgcacgccgctagacctcaggtgcagctggtggaaagcgggggaggcctggttcagcccggcggcagcctgagactgagctgcgccgctagcggcagaacattcagcaactacaacatgggctggttcagacaagcccctggccagggcctggaattcgtggccgctatcgactggtccggcggcagcccttactacgccgcctccgtgcggggcagattcaccatctctcgggataatagcaagaacaccctctacctgcagatgaatagcctgagagccgaggataccgccgtgtactactgtgccgctcctctgtcttacggcagcacctggctggcagattactggggccagggcaccctggtgacagtgtccagcggcggaggaggcagcggcggaggcggaagcggcggtggtggctctggaggcggcggctccggcggtggcggcagtgatatccagatgacccagaccacttccagcctgtctgcctccctgggcgacagggtgactatcagctgccgcgccagccaggatatttcaaaatacctgaattggtaccagcagaagcccgacggcacagtgaagctgctgatctaccacaccagtcgcctgcacagcggcgtgcccagcaggttcagcggcagcggatccggcacagactacagcctgaccatcagcaacctggagcaggaggatatcgcaacttatttttgccagcagggcaatacactgccttacaccttcggcggcggcaccaagctggaaatcaccggcagcacaagtggctccggcaaaccaggcagcggagagggcagcacaaagggcgaggtgaaactgcaggagagcggccccggcctggtggcccccagccagtctctgagcgtgacctgcaccgtgtccggcgtgtccctgcctgactacggggtgagctggatcaggcagccccccaggaaaggcttggaatggctgggcgtgatctggggcagcgagacaacctattataactctgccctgaagagcagactgaccatcatcaaagacaatagcaaaagccaggtgttcctgaagatgaattcactgcagactgacgatactgccatctattattgtgccaaacactactactatggcggatcctatgccatggattactggggccagggcacctcagtgaccgtgtcctcggccgctgctattgaagtgatgtatccacccccttacctggacaacgagaaatcaaacggcactattatccacgtgaagggaaagcacctgtgcccctcccctctgtttcccggcccaagtaagcccttttgggtgctggtggtggtcgggggcgtgctggcctgttattccctgctggtcacagtggctttcatcatcttctgggtgcgcagcaagaggtccagactgctgcactctgactacatgaacatgactcccaggaggccaggccctactagaaaacactaccagccctacgctcctcctagagacttcgccgcctacaggtccagggtcaagttttccagaagcgctgacgctcccgcttaccagcagggccaaaatcagctctataacgaactgaatctcggcaggcgcgaggaatatgacgtgctggataagaggcggggacgcgaccctgaaatgggaggaaagcctcggcggaaaaacccacaagaaggactttacaacgaactccaaaaggataagatggctgaagcctactctgagattggcatgaaaggagaacgtcggagaggaaaaggccacgacggactctatcagggactgtctacagccacaaaagacacatacgacgcactccatatgcaggctctcccacctagaagagcaaagagatccggaagcggcgaaggcagaggatcactgcttacatgcggcgacgtggaagagaaccctggacctatggatatgagagtgccagcccagctgctgggcctgctgctgctgtggctgagaggcgccagatgcgagttcaagcctctgccagaggtgactgatgagtacgacatcgaggtgatgtacccccctccttacctggacaacgagaagtccaacggcaccattatccacgtgaaaggcaagcacctgtgccccagccctctgttccccggcccttctaaaccgttctgggttctggtggtcgtgggcggcgtactggcttgctactctctgctggtcacagtggctttcatcatcttctgggtgaaaagaggcagaaagaaactgctgtacatctttaagcagccattcatgcggccagtgcagaccacccaggaggaggacggctgctcttgtcgctttcccgaggaggaggagggcggatgtgagctgagggtgaagtttagcagatccgctgatgcccctgcctatcagcagggacagaaccagctgtacaacgagctgaacctggggagaagagaagagtacgatgtgctggacaagcggagaggcagagatcctgagatgggcggcaagcccagacggaagaatcctcaagagggcctgtacaatgaactgcagaaagacaagatggccgaggcctacagcgagatcggaatgaagggcgagcgcagaagaggcaagggacacgatggactgtaccagggcctgagcaccgccaccaaggatacctatgatgccctgcacatgcaggccctgcctccaagataa

SEQ ID NO: 70 - DNA, 2655 bp, synthetic construct
  source 1..2655: mol_type = other DNA; note = chimeric antigen receptor
atggcccttccagtgaccgccctgctgctgccactggctctgctgctgcacgccgctagacctcaggtgcagctggtggaaagcgggggaggcctggttcagcccggcggcagcctgagactgagctgcgccgctagcggcagaacattcagcaactacaacatgggctggttcagacaagcccctggccagggcctggaattcgtggccgctatcgactggtccggcggcagcccttactacgccgcctccgtgcggggcagattcaccatctctcgggataatagcaagaacaccctctacctgcagatgaatagcctgagagccgaggataccgccgtgtactactgtgccgctcctctgtcttacggcagcacctggctggcagattactggggccagggcaccctggtgacagtgtccagcggcggaggaggcagcggcggaggcggaagcggcggtggtggctctggaggcggcggctccggcggtggcggcagtgatatccagatgacccagaccacttccagcctgtctgcctccctgggcgacagggtgactatcagctgccgcgccagccaggatatttcaaaatacctgaattggtaccagcagaagcccgacggcacagtgaagctgctgatctaccacaccagtcgcctgcacagcggcgtgcccagcaggttcagcggcagcggatccggcacagactacagcctgaccatcagcaacctggagcaggaggatatcgcaacttatttttgccagcagggcaatacactgccttacaccttcggcggcggcaccaagctggaaatcaccggcagcacaagtggctccggcaaaccaggcagcggagagggcagcacaaagggcgaggtgaaactgcaggagagcggccccggcctggtggcccccagccagtctctgagcgtgacctgcaccgtgtccggcgtgtccctgcctgactacggggtgagctggatcaggcagccccccaggaaaggcttggaatggctgggcgtgatctggggcagcgagacaacctattataactctgccctgaagagcagactgaccatcatcaaagacaatagcaaaagccaggtgttcctgaagatgaattcactgcagactgacgatactgccatctattattgtgccaaacactactactatggcggatcctatgccatggattactggggccagggcacctcagtgaccgtgtcctcgattgaagtgatgtatccacccccttacctggacaacgagaaatcaaacggcactattatccacgtgaagggaaagcacctgtgcccctcccctctgtttcccggcccaagtaagcccttttgggtgctggtggtggtcgggggcgtgctggcctgttattccctgctggtcacagtggctttcatcatcttctgggtgcgcagcaagaggtccagactgctgcactctgactacatgaacatgactcccaggaggccaggccctactagaaaacactaccagccctacgctcctcctagagacttcgccgcctacaggtccagggtcaagttttccagaagcgctgacgctcccgcttaccagcagggccaaaatcagctctataacgaactgaatctcggcaggcgcgaggaatatgacgtgctggataagaggcggggacgcgaccctgaaatgggaggaaagcctcggcggaaaaacccacaagaaggactttacaacgaactccaaaaggataagatggctgaagcctactctgagattggcatgaaaggagaacgtcggagaggaaaaggccacgacggactctatcagggactgtctacagccacaaaagacacatacgacgcactccatatgcaggctctcccacctagaagagcaaagagatccggaagcggcgaaggcagaggatcactgcttacatgcggcgacgtggaagagaaccctggacctatggatatgagagtgccagcccagctgctgggcctgctgctgctgtggctgagaggcgccagatgcgagttcaagcctctgccagaggtgactgatgagtacgcagccgctgaatcaaagtacggccctccttgtccaccctgtccaatctacatttgggcccccctggccgggacatgcggcgtgctcctgctgtctctggtgatcaccctgtactgtaaaagaggcagaaagaaactgctgtacatctttaagcagccattcatgcggccagtgcagaccacccaggaggaggacggctgctcttgtcgctttcccgaggaggaggagggcggatgtgagctgagggtgaagtttagcagatccgctgatgcccctgcctatcagcagggacagaaccagctgtacaacgagctgaacctggggagaagagaagagtacgatgtgctggacaagcggagaggcagagatcctgagatgggcggcaagcccagacggaagaatcctcaagagggcctgtacaatgaactgcagaaagacaagatggccgaggcctacagcgagatcggaatgaagggcgagcgcagaagaggcaagggacacgatggactgtaccagggcctgagcaccgccaccaaggatacctatgatgccctgcacatgcaggccctgcctccaagataa